European Patent Specification EP 4 213 999 B1, published October 29, 2025. Title: COMPOUNDS FOR USE IN SYSTEM SUITABILITY TESTING OF INERT LC SYSTEMS AND COLUMNS. Applicant: WATERS TECHNOLOGIES CORPORATION. The sequence listing filed with the application follows.

SEQUENCE LISTING (2 sequences)

SEQ ID NO: 1 - protein, 10 aa, Artificial Sequence
  Description of Artificial Sequence: Synthetic peptide
  MOD_RES (6)..(6): Phosphothreonine
  MOD_RES (8)..(8): Phosphothreonine
GEGWGTGTGK

SEQ ID NO: 2 - protein, 10 aa, Artificial Sequence
  Description of Artificial Sequence: Synthetic peptide
GEGWGTGTGK